European Patent Specification EP 3 955 002 B1, published April 17, 2024. Title: METHOD FOR CONTROLLING SPEED OF POLYPEPTIDE PASSING THROUGH NANOPORE AND USE THEREOF. Applicant: TSINGHUA UNIVERSITY. The sequence listing filed with the application follows.

SEQUENCE LISTING (5 sequences)

SEQ ID NO: 1 - DNA, 99 bp, Artificial Sequence
  ssDNA
caagaatacctttttttttccttttttttcctctaccacttttcagatctcactatcgcattctcatgcaggtcgtagcttttttcttttttcatcatc

SEQ ID NO: 2 - DNA, 75 bp, Artificial Sequence
  ssDNA-R
tttttttttttttttgctacgacctgcatgagaattttttttttttttttttttttttttttttttttttttttt

SEQ ID NO: 3 - protein, 60 aa, Artificial Sequence
  EGSLFL-60C
EEEEGEEEEGGEEEGGEEESSEEEEGGEEELFEEGGGGEEEESSSSEEEELLEEEEEEEC

SEQ ID NO: 4 - protein, 60 aa, Artificial Sequence
  EDSLFYD-60C
EDEDEEEDYDDDEEEDEEDEVEEEEEYGEVVGELGGGGSHHDHHSSSGSEEEYEEDDDDC

SEQ ID NO: 5 - protein, 30 aa, Artificial Sequence
  E29C
EEEEEEEEEEEEEEEEEEEEEEEEEEEEEC